European Patent Specification EP 3 426 241 B1, published June 12, 2024. Title: METHODS OF DIAGNOSING CANCER. Applicant: Agency for Science, Technology and Research. The sequence listing filed with the application follows.

SEQUENCE LISTING (56 sequences)

SEQ ID NO: 1 - DNA, 20 bp, Artificial Sequence
  ABAT Primer 1
gaggccgtgcactttttctg

SEQ ID NO: 2 - DNA, 20 bp, Artificial Sequence
  ABAT Primer 2
ccagagccggatggttgtaa

SEQ ID NO: 3 - DNA, 20 bp, Artificial Sequence
  ACAA1 Primer 1
acagtgttcatcgggactgc

SEQ ID NO: 4 - DNA, 21 bp, Artificial Sequence
  ACAA1 Primer 2
agatattcccagggttcccca

SEQ ID NO: 5 - DNA, 20 bp, Artificial Sequence
  ACAA2 Primer 1
acataacttcacgcccctgg

SEQ ID NO: 6 - DNA, 20 bp, Artificial Sequence
  ACAA2 Primer 2
gaggggcaaaagcttcgttc

SEQ ID NO: 7 - DNA, 20 bp, Artificial Sequence
  ACADS Primer 1
ttgccgagaaggagttggtc

SEQ ID NO: 8 - DNA, 20 bp, Artificial Sequence
  ACADS Primer 2
aggtaatccaagcctgcacc

SEQ ID NO: 9 - DNA, 20 bp, Artificial Sequence
  ACADSB Primer 1
ggactggcccaaggatgttt

SEQ ID NO: 10 - DNA, 20 bp, Artificial Sequence
  ACADSB Primer 2
cgagcctagcagcgttgtat

SEQ ID NO: 11 - DNA, 20 bp, Artificial Sequence
  ALDH6A1 Primer 1
gcgtgggcagacacatctat

SEQ ID NO: 12 - DNA, 20 bp, Artificial Sequence
  ALDH6A1 Primer 2
ctcccagcatgagggatgtc

SEQ ID NO: 13 - DNA, 20 bp, Artificial Sequence
  AOX1 Primer 1
tacgtgaatggccagaaggt

SEQ ID NO: 14 - DNA, 20 bp, Artificial Sequence
  AOX1 Primer 2
ggatgatgcctgatcgcctt

SEQ ID NO: 15 - DNA, 20 bp, Artificial Sequence
  BCKDHA Primer 1
gacctggtgtttggccagta

SEQ ID NO: 16 - DNA, 20 bp, Artificial Sequence
  BCKDHA Primer 2
gccgtagtgaacaggcatct

SEQ ID NO: 17 - DNA, 20 bp, Artificial Sequence
  ECHS1 Primer 1
ctcttggtgggggttgtgaa

SEQ ID NO: 18 - DNA, 20 bp, Artificial Sequence
  ECHS1 Primer 2
ttgctagcgatttgccgact

SEQ ID NO: 19 - DNA, 19 bp, Artificial Sequence
  HIBCH Primer 1
aggcgtcataacgctcaac

SEQ ID NO: 20 - DNA, 20 bp, Artificial Sequence
  HIBCH Primer 2
tcctccggctccctttatga

SEQ ID NO: 21 - DNA, 20 bp, Artificial Sequence
  HMGCS2 Primer 1
gcccaaacgtctagactccc

SEQ ID NO: 22 - DNA, 20 bp, Artificial Sequence
  HMGCS2 Primer 2
ctccattagacgggacaccg

SEQ ID NO: 23 - DNA, 20 bp, Artificial Sequence
  MCCC1 Primer 1
tggggtagcccgtaaatcca

SEQ ID NO: 24 - DNA, 20 bp, Artificial Sequence
  MCCC1 Primer 2
gagctccttctgcactcact

SEQ ID NO: 25 - DNA, 23 bp, Artificial Sequence
  beta-ACTIN Primer 1
caaggtcatccatgacaactttg

SEQ ID NO: 26 - DNA, 20 bp, Artificial Sequence
  beta-ACTIN Primer 2
ggccatccacagtcttctgg

SEQ ID NO: 27 - DNA, 23 bp, Artificial Sequence
  GAPDH Primer 1
caaggtcatccatgacaactttg

SEQ ID NO: 28 - DNA, 20 bp, Artificial Sequence
  GAPDH Primer 2
ggccatccacagtcttctgg

SEQ ID NO: 29 - DNA, 20 bp, Artificial Sequence
  ABAT Primer 3
gaggccgtgcactttttctg

SEQ ID NO: 30 - DNA, 20 bp, Artificial Sequence
  ABAT Primer 4
cgcgttttgaggctgttgaa

SEQ ID NO: 31 - DNA, 20 bp, Artificial Sequence
  ACAA1 Primer 3
ttacgacattggcatggcct

SEQ ID NO: 32 - DNA, 20 bp, Artificial Sequence
  ACAA1 Primer 4
cagccacattctccgaggtt

SEQ ID NO: 33 - DNA, 20 bp, Artificial Sequence
  ACAA2 Primer 3
ggcaaagttccaccggaaac

SEQ ID NO: 34 - DNA, 20 bp, Artificial Sequence
  ACAA2 Primer 4
actggaaaccagagccacag

SEQ ID NO: 35 - DNA, 20 bp, Artificial Sequence
  ACADS Primer 3
agcctttcaccaaggagtcg

SEQ ID NO: 36 - DNA, 20 bp, Artificial Sequence
  ACADS Primer 4
catctcggtagtagcgctcg

SEQ ID NO: 37 - DNA, 20 bp, Artificial Sequence
  ACADSB Primer 3
ggactggcccaaggatgttt

SEQ ID NO: 38 - DNA, 20 bp, Artificial Sequence
  ACADSB Primer 4
ataaatggcctcccggcttc

SEQ ID NO: 39 - DNA, 20 bp, Artificial Sequence
  ALDH6A1 Primer 3
agtacctggagcaaccatgc

SEQ ID NO: 40 - DNA, 20 bp, Artificial Sequence
  ALDH6A1 Primer 4
cgaagatgtactctcccgcc

SEQ ID NO: 41 - DNA, 21 bp, Artificial Sequence
  AOX1 Primer 3
accgtacctgaggaagaacct

SEQ ID NO: 42 - DNA, 20 bp, Artificial Sequence
  AOX1 Primer 4
tgccctctactgtggtgact

SEQ ID NO: 43 - DNA, 20 bp, Artificial Sequence
  BCKDHA Primer 3
caacgatgtgtttgcggtgt

SEQ ID NO: 44 - DNA, 20 bp, Artificial Sequence
  BCKDHA Primer 4
ttgacctcatccaccgaacg

SEQ ID NO: 45 - DNA, 20 bp, Artificial Sequence
  ECHS1 Primer 3
aggccatccaatgtgcagaa

SEQ ID NO: 46 - DNA, 20 bp, Artificial Sequence
  ECHS1 Primer 4
tccacaaaggcagacatccc

SEQ ID NO: 47 - DNA, 25 bp, Artificial Sequence
  HIBCH Primer 3
tggaacagattaagttctcattgac

SEQ ID NO: 48 - DNA, 20 bp, Artificial Sequence
  HIBCH Primer 4
tatggtgtgctgacccttgc

SEQ ID NO: 49 - DNA, 20 bp, Artificial Sequence
  HMGCS2 Primer 3
gcccaaacgtctagactccc

SEQ ID NO: 50 - DNA, 20 bp, Artificial Sequence
  HMGCS2 Primer 4
cgggcatattttctgcggtg

SEQ ID NO: 51 - DNA, 20 bp, Artificial Sequence
  MCCC1 Primer 3
aaggcatgtggaagtccagg

SEQ ID NO: 52 - DNA, 20 bp, Artificial Sequence
  MCCC1 Primer 4
caggatcaataccaggcgct

SEQ ID NO: 53 - DNA, 23 bp, Artificial Sequence
  beta-ACTIN Primer 3
caaggtcatccatgacaactttg

SEQ ID NO: 54 - DNA, 20 bp, Artificial Sequence
  beta-ACTIN Primer 4
ggccatccacagtcttctga

SEQ ID NO: 55 - DNA, 23 bp, Artificial Sequence
  GAPDH Primer 3
caaggtcatccatgacaactttg

SEQ ID NO: 56 - DNA, 20 bp, Artificial Sequence
  GAPDH Primer 4
ggccatccacagtcttctga